European Patent Specification EP 3 295 345 B1, published January 25, 2023. Title: BARCODE SEQUENCES, AND RELATED SYSTEMS AND METHODS. Applicant: LIFE TECHNOLOGIES CORPORATION. The sequence listing filed with the application follows.

SEQUENCE LISTING (79 sequences)

SEQ ID NO: 1 - DNA, 14 bp, Artificial Sequence
  source: /note="Description of Artificial Sequence: Synthetic oligonucleotide"
tcagtcctcgaatc

SEQ ID NO: 2 - DNA, 14 bp, Artificial Sequence
  source: /note="Description of Artificial Sequence: Synthetic oligonucleotide"
tcagcttgcggatc

SEQ ID NO: 3 - DNA, 14 bp, Artificial Sequence
  source: /note="Description of Artificial Sequence: Synthetic oligonucleotide"
tcagtctaacggac

SEQ ID NO: 4 - DNA, 14 bp, Artificial Sequence
  source: /note="Description of Artificial Sequence: Synthetic oligonucleotide"
tcagttcttagcgc

SEQ ID NO: 5 - DNA, 14 bp, Artificial Sequence
  source: /note="Description of Artificial Sequence: Synthetic oligonucleotide"
tcagtgagcggaac

SEQ ID NO: 6 - DNA, 14 bp, Artificial Sequence
  source: /note="Description of Artificial Sequence: Synthetic oligonucleotide"
tcagttaagcggtc

SEQ ID NO: 7 - DNA, 14 bp, Artificial Sequence
  source: /note="Description of Artificial Sequence: Synthetic oligonucleotide"
tcagctgaccgaac

SEQ ID NO: 8 - DNA, 14 bp, Artificial Sequence
  source: /note="Description of Artificial Sequence: Synthetic oligonucleotide"
tcagtctagaggtc

SEQ ID NO: 9 - DNA, 14 bp, Artificial Sequence
  source: /note="Description of Artificial Sequence: Synthetic oligonucleotide"
tcagaagaggattc

SEQ ID NO: 10 - DNA, 10 bp, Artificial Sequence
  source: /note="Description of Artificial Sequence: Synthetic oligonucleotide"
tcctcgaatc

SEQ ID NO: 11 - DNA, 10 bp, Artificial Sequence
  source: /note="Description of Artificial Sequence: Synthetic oligonucleotide"
cttgcggatc

SEQ ID NO: 12 - DNA, 10 bp, Artificial Sequence
  source: /note="Description of Artificial Sequence: Synthetic oligonucleotide"
tctaacggac

SEQ ID NO: 13 - DNA, 10 bp, Artificial Sequence
  source: /note="Description of Artificial Sequence: Synthetic oligonucleotide"
ttcttagcgc

SEQ ID NO: 14 - DNA, 10 bp, Artificial Sequence
  source: /note="Description of Artificial Sequence: Synthetic oligonucleotide"
tgagcggaac

SEQ ID NO: 15 - DNA, 10 bp, Artificial Sequence
  source: /note="Description of Artificial Sequence: Synthetic oligonucleotide"
ttaagcggtc

SEQ ID NO: 16 - DNA, 10 bp, Artificial Sequence
  source: /note="Description of Artificial Sequence: Synthetic oligonucleotide"
ctgaccgaac

SEQ ID NO: 17 - DNA, 10 bp, Artificial Sequence
  source: /note="Description of Artificial Sequence: Synthetic oligonucleotide"
tctagaggtc

SEQ ID NO: 18 - DNA, 10 bp, Artificial Sequence
  source: /note="Description of Artificial Sequence: Synthetic oligonucleotide"
aagaggattc

SEQ ID NO: 19 - DNA, 14 bp, Artificial Sequence
  source: /note="Description of Artificial Sequence: Synthetic oligonucleotide"
tctgagcatcgatc

SEQ ID NO: 20 - DNA, 14 bp, Artificial Sequence
  source: /note="Description of Artificial Sequence: Synthetic oligonucleotide"
ttccggaggatgcc

SEQ ID NO: 21 - DNA, 14 bp, Artificial Sequence
  source: /note="Description of Artificial Sequence: Synthetic oligonucleotide"
ttgaggccaagtcc

SEQ ID NO: 22 - DNA, 12 bp, Artificial Sequence
  source: /note="Description of Artificial Sequence: Synthetic oligonucleotide"
gaccaccggttc

SEQ ID NO: 23 - DNA, 14 bp, Artificial Sequence
  source: /note="Description of Artificial Sequence: Synthetic oligonucleotide"
gtggacctccgttc

SEQ ID NO: 24 - DNA, 14 bp, Artificial Sequence
  source: /note="Description of Artificial Sequence: Synthetic oligonucleotide"
tggaccacgaattc

SEQ ID NO: 25 - DNA, 14 bp, Artificial Sequence
  source: /note="Description of Artificial Sequence: Synthetic oligonucleotide"
ttctggacatccgc

SEQ ID NO: 26 - DNA, 14 bp, Artificial Sequence
  source: /note="Description of Artificial Sequence: Synthetic oligonucleotide"
ttaggcctccattc

SEQ ID NO: 27 - DNA, 14 bp, Artificial Sequence
  source: /note="Description of Artificial Sequence: Synthetic oligonucleotide"
gttgaggaaccacc

SEQ ID NO: 28 - DNA, 14 bp, Artificial Sequence
  source: /note="Description of Artificial Sequence: Synthetic oligonucleotide"
ccggacaagaattc

SEQ ID NO: 29 - DNA, 14 bp, Artificial Sequence
  source: /note="Description of Artificial Sequence: Synthetic oligonucleotide"
cggagttccggttc

SEQ ID NO: 30 - DNA, 14 bp, Artificial Sequence
  source: /note="Description of Artificial Sequence: Synthetic oligonucleotide"
gtccaccaaccacc

SEQ ID NO: 31 - DNA, 14 bp, Artificial Sequence
  source: /note="Description of Artificial Sequence: Synthetic oligonucleotide"
gttccagccatctc

SEQ ID NO: 32 - DNA, 12 bp, Artificial Sequence
  source: /note="Description of Artificial Sequence: Synthetic oligonucleotide"
gttagcggattc

SEQ ID NO: 33 - DNA, 12 bp, Artificial Sequence
  source: /note="Description of Artificial Sequence: Synthetic oligonucleotide"
gccacaacttcc

SEQ ID NO: 34 - DNA, 14 bp, Artificial Sequence
  source: /note="Description of Artificial Sequence: Synthetic oligonucleotide"
gttccttagaagac

SEQ ID NO: 35 - DNA, 14 bp, Artificial Sequence
  source: /note="Description of Artificial Sequence: Synthetic oligonucleotide"
gccagcaccaattc

SEQ ID NO: 36 - DNA, 14 bp, Artificial Sequence
  source: /note="Description of Artificial Sequence: Synthetic oligonucleotide"
gcttggagccgttc

SEQ ID NO: 37 - DNA, 14 bp, Artificial Sequence
  source: /note="Description of Artificial Sequence: Synthetic oligonucleotide"
tccaggcaccttcc

SEQ ID NO: 38 - DNA, 12 bp, Artificial Sequence
  source: /note="Description of Artificial Sequence: Synthetic oligonucleotide"
gttcctacgttc

SEQ ID NO: 39 - DNA, 14 bp, Artificial Sequence
  source: /note="Description of Artificial Sequence: Synthetic oligonucleotide"
ccagaacggaatcc

SEQ ID NO: 40 - DNA, 12 bp, Artificial Sequence
  source: /note="Description of Artificial Sequence: Synthetic oligonucleotide"
gtcaggaccaac

SEQ ID NO: 41 - DNA, 14 bp, Artificial Sequence
  source: /note="Description of Artificial Sequence: Synthetic oligonucleotide"
cttaccatccttcc

SEQ ID NO: 42 - DNA, 12 bp, Artificial Sequence
  source: /note="Description of Artificial Sequence: Synthetic oligonucleotide"
gctgacaccacc

SEQ ID NO: 43 - DNA, 12 bp, Artificial Sequence
  source: /note="Description of Artificial Sequence: Synthetic oligonucleotide"
tcaccaacggac

SEQ ID NO: 44 - DNA, 14 bp, Artificial Sequence
  source: /note="Description of Artificial Sequence: Synthetic oligonucleotide"
ctgagaatccaacc

SEQ ID NO: 45 - DNA, 14 bp, Artificial Sequence
  source: /note="Description of Artificial Sequence: Synthetic oligonucleotide"
ttcctacaatctcc

SEQ ID NO: 46 - DNA, 14 bp, Artificial Sequence
  source: /note="Description of Artificial Sequence: Synthetic oligonucleotide"
gtcttgacaagaac

SEQ ID NO: 47 - DNA, 14 bp, Artificial Sequence
  source: /note="Description of Artificial Sequence: Synthetic oligonucleotide"
gttcttagagaacc

SEQ ID NO: 48 - DNA, 12 bp, Artificial Sequence
  source: /note="Description of Artificial Sequence: Synthetic oligonucleotide"
gtccaggaggtc

SEQ ID NO: 49 - DNA, 14 bp, Artificial Sequence
  source: /note="Description of Artificial Sequence: Synthetic oligonucleotide"
tcggaccaattgcc

SEQ ID NO: 50 - DNA, 14 bp, Artificial Sequence
  source: /note="Description of Artificial Sequence: Synthetic oligonucleotide"
ccttaccaataacc

SEQ ID NO: 51 - DNA, 14 bp, Artificial Sequence
  source: /note="Description of Artificial Sequence: Synthetic oligonucleotide"
tcgaggccatcgac

SEQ ID NO: 52 - DNA, 14 bp, Artificial Sequence
  source: /note="Description of Artificial Sequence: Synthetic oligonucleotide"
ttccttaccttatc

SEQ ID NO: 53 - DNA, 12 bp, Artificial Sequence
  source: /note="Description of Artificial Sequence: Synthetic oligonucleotide"
ttctgagccgac

SEQ ID NO: 54 - DNA, 14 bp, Artificial Sequence
  source: /note="Description of Artificial Sequence: Synthetic oligonucleotide"
gtcctaccaatgac

SEQ ID NO: 55 - DNA, 14 bp, Artificial Sequence
  source: /note="Description of Artificial Sequence: Synthetic oligonucleotide"
tagccaattgaacc

SEQ ID NO: 56 - DNA, 14 bp, Artificial Sequence
  source: /note="Description of Artificial Sequence: Synthetic oligonucleotide"
gccttagcaacacc

SEQ ID NO: 57 - DNA, 14 bp, Artificial Sequence
  source: /note="Description of Artificial Sequence: Synthetic oligonucleotide"
gtcctgagcagaac

SEQ ID NO: 58 - DNA, 12 bp, Artificial Sequence
  source: /note="Description of Artificial Sequence: Synthetic oligonucleotide"
gtctacctcggc

SEQ ID NO: 59 - DNA, 14 bp, Artificial Sequence
  source: /note="Description of Artificial Sequence: Synthetic oligonucleotide"
gtctgaccggatcc

SEQ ID NO: 60 - DNA, 14 bp, Artificial Sequence
  source: /note="Description of Artificial Sequence: Synthetic oligonucleotide"
ccagaattcggacc

SEQ ID NO: 61 - DNA, 14 bp, Artificial Sequence
  source: /note="Description of Artificial Sequence: Synthetic oligonucleotide"
ttccggagttcatc

SEQ ID NO: 62 - DNA, 14 bp, Artificial Sequence
  source: /note="Description of Artificial Sequence: Synthetic oligonucleotide"
ccttagatccttcc

SEQ ID NO: 63 - DNA, 14 bp, Artificial Sequence
  source: /note="Description of Artificial Sequence: Synthetic oligonucleotide"
gccttaggatcgcc

SEQ ID NO: 64 - DNA, 14 bp, Artificial Sequence
  source: /note="Description of Artificial Sequence: Synthetic oligonucleotide"
gccaggattggtcc

SEQ ID NO: 65 - DNA, 14 bp, Artificial Sequence
  source: /note="Description of Artificial Sequence: Synthetic oligonucleotide"
gtccggagatgaac

SEQ ID NO: 66 - DNA, 14 bp, Artificial Sequence
  source: /note="Description of Artificial Sequence: Synthetic oligonucleotide"
gccttattccaacc

SEQ ID NO: 67 - DNA, 14 bp, Artificial Sequence
  source: /note="Description of Artificial Sequence: Synthetic oligonucleotide"
gttctaggattcac

SEQ ID NO: 68 - DNA, 14 bp, Artificial Sequence
  source: /note="Description of Artificial Sequence: Synthetic oligonucleotide"
tcctagtccggtcc

SEQ ID NO: 69 - DNA, 14 bp, Artificial Sequence
  source: /note="Description of Artificial Sequence: Synthetic oligonucleotide"
gtcttggagttaac

SEQ ID NO: 70 - DNA, 12 bp, Artificial Sequence
  source: /note="Description of Artificial Sequence: Synthetic oligonucleotide"
gttctatcgttc

SEQ ID NO: 71 - DNA, 12 bp, Artificial Sequence
  source: /note="Description of Artificial Sequence: Synthetic oligonucleotide"
ttcgagtgttcc

SEQ ID NO: 72 - DNA, 12 bp, Artificial Sequence
  source: /note="Description of Artificial Sequence: Synthetic oligonucleotide"
tcttgattggtc

SEQ ID NO: 73 - DNA, 14 bp, Artificial Sequence
  source: /note="Description of Artificial Sequence: Synthetic oligonucleotide"
gcttactccggtcc

SEQ ID NO: 74 - DNA, 12 bp, Artificial Sequence
  source: /note="Description of Artificial Sequence: Synthetic oligonucleotide"
gattcggattcc

SEQ ID NO: 75 - DNA, 14 bp, Artificial Sequence
  source: /note="Description of Artificial Sequence: Synthetic oligonucleotide"
gttcctgagttctc

SEQ ID NO: 76 - DNA, 14 bp, Artificial Sequence
  source: /note="Description of Artificial Sequence: Synthetic oligonucleotide"
gtcggaccatgaac

SEQ ID NO: 77 - DNA, 12 bp, Artificial Sequence
  source: /note="Description of Artificial Sequence: Synthetic oligonucleotide"
cagatccgttcc

SEQ ID NO: 78 - DNA, 12 bp, Artificial Sequence
  source: /note="Description of Artificial Sequence: Synthetic oligonucleotide"
gttctgacgtcc

SEQ ID NO: 79 - DNA, 14 bp, Artificial Sequence
  source: /note="Description of Artificial Sequence: Synthetic oligonucleotide"
tccgaggatgaatc